European Patent Application EP 4 737 474 A1, published May 6, 2026. Title: SYNTHETIC PEPTIDE, PHARMACEUTICAL COMPOSITION COMPRISING SYNTHETIC PEPTIDE, AND USE OF SYNTHETIC PEPTIDE FOR TREATING AMYLOIDOSIS. Applicant: China Medical University Hospital. Application US. The sequence listing filed with the application follows.

SEQUENCE LISTING (1 sequence)

SEQ ID NO: 1 - protein, 45 aa, synthetic construct
GGGYSKAQKAQAKEAKQAQKAQKAQAKEAKQAQKAQKAQAKQAKQ